European Patent Application EP 4 501 962 A1, published February 5, 2025. Title: 抗CD7纳米抗体、衍生物及其在肿瘤治疗中的应用. Applicant: 河北森朗生物科技有限公司. The sequence listing filed with the application follows.

SEQUENCE LISTING (161 sequences)

SEQ ID NO: 1 - protein, 124 aa, Artificial sequence
QVQLQESGGGLVQPGGSLRLSCTASGLTLGYYAIGWFRQAPGGEREGVSCISAGGTSTLYADSVKGRFTISRDNSKSTVYLQMNSLKPEDTALYTCALRSVRSCSLAQAAFDYWGQGTQVTVSS

SEQ ID NO: 2 - DNA, 372 bp, Artificial sequence
  source 1..372: mol_type = other DNA
caggtgcagctgcaggagtctggaggaggcttggtgcagcctggggggtctctgagactctcctgtacagcctctggattgactctgggttattatgccataggctggttccgccaggccccagggggggagcgtgagggggtctcatgtataagtgctggtggtactagcacactctatgcagactccgtgaagggccgattcaccatctccagagacaactccaagagcacggtgtatctgcaaatgaacagcctgaaacctgaagacacagccctttacacgtgtgcactacgttcagtacgttcgtgctcgctagcacaggctgcgttcgactactggggccagggaacccaggtcaccgtctcctca

SEQ ID NO: 3 - protein, 8 aa, Artificial sequence
GLTLGYYA

SEQ ID NO: 4 - DNA, 24 bp, Artificial sequence
  source 1..24: mol_type = other DNA
ggattgactctgggttattatgcc

SEQ ID NO: 5 - protein, 8 aa, Artificial sequence
ISAGGTST

SEQ ID NO: 6 - DNA, 24 bp, Artificial sequence
  source 1..24: mol_type = other DNA
ataagtgctggtggtactagcaca

SEQ ID NO: 7 - protein, 17 aa, Artificial sequence
ALRSVRSCSLAQAAFDY

SEQ ID NO: 8 - DNA, 51 bp, Artificial sequence
  source 1..51: mol_type = other DNA
gcactacgttcagtacgttcgtgctcgctagcacaggctgcgttcgactac

SEQ ID NO: 9 - protein, 125 aa, Artificial sequence
QVQLQESGGGSVQAGGSLRLSCAASGRVFSSDAMGWFRQAPGNEREFVAAIIWSGSSTHYADSVKGRFTISRDNAKNTGYLQMNSLKPEDTAVYYCAVDTRPPYGLRNANRYDYWGQGTQVTVSS

SEQ ID NO: 10 - DNA, 375 bp, Artificial sequence
  source 1..375: mol_type = other DNA
caggtgcagctgcaggagtctggaggaggatcggtgcaggctgggggctctctgagactctcctgtgcagcctctggacgcgtcttcagtagcgatgccatgggctggttccgccaggctccagggaacgagcgtgagtttgtagcagctattatctggagtggtagtagcacacactatgcagactccgtgaagggccgattcaccatctccagagacaacgccaagaacacggggtatctgcaaatgaacagcctgaaacctgaggacacggccgtttattactgtgcagtagacactcgccctccatacggattgaggaacgcaaaccggtatgactactggggccaggggacccaggtcaccgtctcctca

SEQ ID NO: 11 - protein, 8 aa, Artificial sequence
GRVFSSDA

SEQ ID NO: 12 - DNA, 24 bp, Artificial sequence
  source 1..24: mol_type = other DNA
ggacgcgtcttcagtagcgatgcc

SEQ ID NO: 13 - protein, 8 aa, Artificial sequence
IIWSGSST

SEQ ID NO: 14 - DNA, 24 bp, Artificial sequence
  source 1..24: mol_type = other DNA
attatctggagtggtagtagcaca

SEQ ID NO: 15 - protein, 18 aa, Artificial sequence
AVDTRPPYGLRNANRYDY

SEQ ID NO: 16 - DNA, 54 bp, Artificial sequence
  source 1..54: mol_type = other DNA
gcagtagacactcgccctccatacggattgaggaacgcaaaccggtatgactac

SEQ ID NO: 17 - protein, 114 aa, Artificial sequence
QVQLQESGGGLVQPGGSLRLSCVDSRSVFRAIAMGWYRQAPGKQRELVARISSGGNTNYADFVKGRFTITRDNAKNTLYLQMNSLKPEDTAVYYCNREPPDYVWGQGTQVTVSS

SEQ ID NO: 18 - DNA, 342 bp, Artificial sequence
  source 1..342: mol_type = other DNA
caggtgcagctgcaggagtctgggggaggcttggtgcagcctggggggtctctgagactctcctgtgtagactctagaagcgtcttcagagccattgccatgggctggtaccgccaggctccagggaagcagcgcgagttggtcgcacgtattagtagtggtggaaacacaaactatgcagacttcgtgaagggccgattcaccatcaccagagacaacgccaagaacacgctgtatctgcaaatgaacagcctgaaacctgaggacacggccgtctattactgcaatcgagaaccccctgactacgtatggggccaggggacccaggtcaccgtctcctca

SEQ ID NO: 19 - protein, 8 aa, Artificial sequence
RSVFRAIA

SEQ ID NO: 20 - DNA, 24 bp, Artificial sequence
  source 1..24: mol_type = other DNA
agaagcgtcttcagagccattgcc

SEQ ID NO: 21 - protein, 7 aa, Artificial sequence
ISSGGNT

SEQ ID NO: 22 - DNA, 21 bp, Artificial sequence
  source 1..21: mol_type = other DNA
attagtagtggtggaaacaca

SEQ ID NO: 23 - protein, 8 aa, Artificial sequence
NREPPDYV

SEQ ID NO: 24 - DNA, 24 bp, Artificial sequence
  source 1..24: mol_type = other DNA
aatcgagaaccccctgactacgta

SEQ ID NO: 25 - protein, 124 aa, Artificial sequence
QVQLQESGGGLVQAGGSLRLSCAASGRTFSSYNMGWFRQAPGAEREFVAAISRGGGSTYYADSVKGRFTISRDNAKNTVYLQMNSLRPEDTAVYYCADSGARAYSGSYLDFGSWGQGTQVTVSS

SEQ ID NO: 26 - DNA, 372 bp, Artificial sequence
  source 1..372: mol_type = other DNA
caggtgcagctgcaggagtctggaggaggattggtgcaggctgggggctctctgagactctcctgtgcagcctctggacgcaccttcagtagctataacatgggctggttccgccaggctccaggggcggagcgcgagtttgtagcagctattagccggggtggtggtagtacatactatgcagactccgtgaagggccgattcaccatctccagagacaacgccaagaacacggtgtatctgcaaatgaacagcctgcgacctgaggacacggccgtttattactgtgcagactcaggagctcgagcctatagtggtagttacctcgactttggttcctggggccaggggacccaggtcaccgtctcctca

SEQ ID NO: 27 - protein, 8 aa, Artificial sequence
GRTFSSYN

SEQ ID NO: 28 - DNA, 24 bp, Artificial sequence
  source 1..24: mol_type = other DNA
ggacgcaccttcagtagctataac

SEQ ID NO: 29 - protein, 8 aa, Artificial sequence
ISRGGGST

SEQ ID NO: 30 - DNA, 24 bp, Artificial sequence
  source 1..24: mol_type = other DNA
attagccggggtggtggtagtaca

SEQ ID NO: 31 - protein, 17 aa, Artificial sequence
ADSGARAYSGSYLDFGS

SEQ ID NO: 32 - DNA, 51 bp, Artificial sequence
  source 1..51: mol_type = other DNA
gcagactcaggagctcgagcctatagtggtagttacctcgactttggttcc

SEQ ID NO: 33 - protein, 124 aa, Artificial sequence
QVQLQESGGGLVQAGGSLRLSCAASGRTFSSYVMKWFRQAPGKGREFVAGISWSGSLTSYSDSVKGRFTISRDNAKNTVYLQMNSLKPEDTAVYYCAAGEAATMSDTDYGMDYWGKGTQVTVSS

SEQ ID NO: 34 - DNA, 372 bp, Artificial sequence
  source 1..372: mol_type = other DNA
caggtgcagctgcaggagtctgggggaggattggtgcaggctgggggctctctgagactctcctgtgcagcctctggacgcaccttcagtagttatgtcatgaaatggtttcgccaggctccaggaaaggggcgagaatttgtagctggtattagttggagtggtagtcttacaagctattcagactccgtgaagggccgattcactatctccagagacaacgccaagaacacggtgtatctgcaaatgaacagcctgaaacctgaggacacggccgtttattactgtgcggccggagaagccgcgactatgtctgataccgactacggcatggactactggggcaaagggacccaggtcaccgtctcctca

SEQ ID NO: 35 - protein, 8 aa, Artificial sequence
GRTFSSYV

SEQ ID NO: 36 - DNA, 24 bp, Artificial sequence
  source 1..24: mol_type = other DNA
ggacgcaccttcagtagttatgtc

SEQ ID NO: 37 - protein, 8 aa, Artificial sequence
ISWSGSLT

SEQ ID NO: 38 - DNA, 24 bp, Artificial sequence
  source 1..24: mol_type = other DNA
attagttggagtggtagtcttaca

SEQ ID NO: 39 - protein, 17 aa, Artificial sequence
AAGEAATMSDTDYGMDY

SEQ ID NO: 40 - DNA, 51 bp, Artificial sequence
  source 1..51: mol_type = other DNA
gcggccggagaagccgcgactatgtctgataccgactacggcatggactac

SEQ ID NO: 41 - protein, 117 aa, Artificial sequence
QVQLQESGGGLVQPGGSLRLSCAASGSIFSIHAMAWYRQAPGKQRELVASITVGGRTNYVDSVLGRFTISRDNAKNTVYLQMNSLKPEDTAVYYCNSLLWAGLRDSWGPGTQVTVSS

SEQ ID NO: 42 - DNA, 351 bp, Artificial sequence
  source 1..351: mol_type = other DNA
caggtgcagctgcaggagtctggaggaggcttggtgcagcctggggggtccctgagactctcctgtgcagcctctggaagcatcttcagtatccatgctatggcctggtaccggcaggctcctgggaagcagcgagaattggtcgcatctattacagtaggtggtaggacaaactatgtagactccgtgctgggccgattcaccatctccagagacaacgccaagaacacggtgtatctgcaaatgaacagcctgaaacctgaggacacggccgtctattactgtaactcactcttatgggccgggctgagggattcctggggtccggggacccaggtcaccgtctcctca

SEQ ID NO: 43 - protein, 8 aa, Artificial sequence
GSIFSIHA

SEQ ID NO: 44 - DNA, 24 bp, Artificial sequence
  source 1..24: mol_type = other DNA
ggaagcatcttcagtatccatgct

SEQ ID NO: 45 - protein, 7 aa, Artificial sequence
ITVGGRT

SEQ ID NO: 46 - DNA, 21 bp, Artificial sequence
  source 1..21: mol_type = other DNA
attacagtaggtggtaggaca

SEQ ID NO: 47 - protein, 11 aa, Artificial sequence
NSLLWAGLRDS

SEQ ID NO: 48 - DNA, 33 bp, Artificial sequence
  source 1..33: mol_type = other DNA
aactcactcttatgggccgggctgagggattcc

SEQ ID NO: 49 - protein, 117 aa, Artificial sequence
QVQLQESGGGLVQPGGSLRLSCVASGSKFSISTMGWYRQAPGKQRDLVASITPGGNTAYAEAVKGRFTISRDNAKNTVYLQMNSLKPEDTAVYYCNDFRLAGLRDYWGQGTQVTVSS

SEQ ID NO: 50 - DNA, 351 bp, Artificial sequence
  source 1..351: mol_type = other DNA
caggtgcagctgcaggagtctggaggaggcttggtgcagcctggggggtctctgagactctcttgtgtagcctctggaagcaagttcagtatcagtaccatgggctggtaccgccaggctccagggaagcagcgcgatttggtcgcatctattacgcctggtggtaacacagcctatgcagaagccgtgaagggccgattcaccatctccagagacaacgccaagaacacggtgtatctgcaaatgaacagcctgaaacctgaggacacggccgtctattactgtaatgacttccgtctagctggtctgagggactactggggccaggggacccaggtcaccgtctcctca

SEQ ID NO: 51 - protein, 8 aa, Artificial sequence
GSKFSIST

SEQ ID NO: 52 - DNA, 24 bp, Artificial sequence
  source 1..24: mol_type = other DNA
ggaagcaagttcagtatcagtacc

SEQ ID NO: 53 - protein, 7 aa, Artificial sequence
ITPGGNT

SEQ ID NO: 54 - DNA, 21 bp, Artificial sequence
  source 1..21: mol_type = other DNA
attacgcctggtggtaacaca

SEQ ID NO: 55 - protein, 11 aa, Artificial sequence
NDFRLAGLRDY

SEQ ID NO: 56 - DNA, 33 bp, Artificial sequence
  source 1..33: mol_type = other DNA
aatgacttccgtctagctggtctgagggactac

SEQ ID NO: 57 - protein, 124 aa, Artificial sequence
QVQLQESGGGLVQTGGSLRLSCEASERTFSSNAVGWFRQAPGKEREFVAAITWSVGTTYYADSVKGRFTISRDNAKNTVYLQMNSLKPEDTAVYYCAASGARHYSGSYLDFGSWGQGTQVTVSS

SEQ ID NO: 58 - DNA, 372 bp, Artificial sequence
  source 1..372: mol_type = other DNA
caggtgcagctgcaggagtctggaggaggcttggtgcaaactgggggttctctgagactctcctgtgaagcctctgaacgcaccttcagtagcaatgccgtgggctggttccgccaggctccagggaaggagcgtgagtttgtagcagctattacctggagtgttggtaccacatactatgcagactccgtgaagggccgattcaccatctccagagacaacgccaagaacacggtgtatctgcaaatgaacagcctgaaacctgaggacacggccgtttattactgtgcagcctcaggagctcgacactatagtggtagttacctcgactttggttcctggggccaggggacccaggtcaccgtctcctca

SEQ ID NO: 59 - protein, 8 aa, Artificial sequence
ERTFSSNA

SEQ ID NO: 60 - DNA, 24 bp, Artificial sequence
  source 1..24: mol_type = other DNA
gaacgcaccttcagtagcaatgcc

SEQ ID NO: 61 - protein, 8 aa, Artificial sequence
ITWSVGTT

SEQ ID NO: 62 - DNA, 24 bp, Artificial sequence
  source 1..24: mol_type = other DNA
attacctggagtgttggtaccaca

SEQ ID NO: 63 - protein, 17 aa, Artificial sequence
AASGARHYSGSYLDFGS

SEQ ID NO: 64 - DNA, 51 bp, Artificial sequence
  source 1..51: mol_type = other DNA
gcagcctcaggagctcgacactatagtggtagttacctcgactttggttcc

SEQ ID NO: 65 - protein, 129 aa, Artificial sequence
QVQLQESGGGLVQPGGSLRLSCAASGSTLDYYAIGWFRQAPGKEREGISCISNSGGMTNYADSVKGRFTISRDNAKNTVYLQMNSLKPEDTAVYYCAAGPAWSYCSGYVPAGLDKFGSWGQGTQVTVSS

SEQ ID NO: 66 - DNA, 387 bp, Artificial sequence
  source 1..387: mol_type = other DNA
caggtgcagctgcaggagtctgggggaggcttggtgcagcctggggggtctctgagactctcctgtgcagcctctggatccactttggattattatgccataggctggttccgccaggccccagggaaggagcgtgagggcatctcatgtattagtaatagtggtggtatgacaaactatgcagactccgtgaagggccgattcaccatctccagagacaacgccaagaacacggtgtatctgcaaatgaacagcctgaaacctgaggacacagccgtttattactgtgcagcaggcccggcgtggtcctactgttcaggctatgtgccggccggcctagataaatttggttcttggggccaggggacccaggtcaccgtctcctca

SEQ ID NO: 67 - protein, 8 aa, Artificial sequence
GSTLDYYA

SEQ ID NO: 68 - DNA, 24 bp, Artificial sequence
  source 1..24: mol_type = other DNA
ggatccactttggattattatgcc

SEQ ID NO: 69 - protein, 8 aa, Artificial sequence
ISNSGGMT

SEQ ID NO: 70 - DNA, 24 bp, Artificial sequence
  source 1..24: mol_type = other DNA
attagtaatagtggtggtatgaca

SEQ ID NO: 71 - protein, 22 aa, Artificial sequence
AAGPAWSYCSGYVPAGLDKFGS

SEQ ID NO: 72 - DNA, 66 bp, Artificial sequence
  source 1..66: mol_type = other DNA
gcagcaggcccggcgtggtcctactgttcaggctatgtgccggccggcctagataaatttggttct

SEQ ID NO: 73 - protein, 125 aa, Artificial sequence
QVQLQESGGGLVQAGGSLNLSCTVYGFTADDYAVGWFRQAPGKGRQGISCLSRKDGSKYVADPVLGRATISSDNTKNTVRLTLSALKPDDTAVYYCAAHRFATFCGTRDYEYDYWGQGTQVTVSS

SEQ ID NO: 74 - DNA, 375 bp, Artificial sequence
  source 1..375: mol_type = other DNA
caggtgcagctgcaggagtctggaggaggcttggtgcaggctgggggctctctgaacctctcctgtacagtctatgggttcactgccgatgactatgccgtaggctggttccgccaggccccagggaagggacgacaagggatctcatgtcttagccgtaaggatggcagcaagtacgtggctgatcccgtgctgggccgagccaccatctccagtgacaacaccaagaacactgtgcgtctgaccctgagcgcattgaaacctgacgatacggccgtctattactgtgcagctcatagatttgcgacattctgtggcacccgtgattatgagtatgactattggggccagggaacccaggtcaccgtctcctca

SEQ ID NO: 75 - protein, 8 aa, Artificial sequence
GFTADDYA

SEQ ID NO: 76 - DNA, 24 bp, Artificial sequence
  source 1..24: mol_type = other DNA
gggttcactgccgatgactatgcc

SEQ ID NO: 77 - protein, 8 aa, Artificial sequence
LSRKDGSK

SEQ ID NO: 78 - DNA, 24 bp, Artificial sequence
  source 1..24: mol_type = other DNA
cttagccgtaaggatggcagcaag

SEQ ID NO: 79 - protein, 18 aa, Artificial sequence
AAHRFATFCGTRDYEYDY

SEQ ID NO: 80 - DNA, 54 bp, Artificial sequence
  source 1..54: mol_type = other DNA
gcagctcatagatttgcgacattctgtggcacccgtgattatgagtatgactat

SEQ ID NO: 81 - protein, 122 aa, Artificial sequence
QVQLQESGGGLVQPGGSLRLSCTASGLTLGYYAIGWFRQAPGKEREFVSTISASGGMTYYADSVKGRFTISRDNAKNTVYLEMNSLKPEDTAVYYCAAEYLGNLRHFRGDHWGKGTQVTVSS

SEQ ID NO: 82 - DNA, 366 bp, Artificial sequence
  source 1..366: mol_type = other DNA
caggtgcagctgcaggagtctgggggaggcttggtgcagcctggggggtctctgagactctcctgtacagcctctggattgactctgggttattatgccataggctggttccgccaggctccagggaaggagcgtgagtttgtgtcgactattagcgcgagtggtggtatgacatactatgcagactccgtgaagggccgattcaccatctccagagacaacgccaagaacacggtgtatctggaaatgaacagcctgaaacctgaggacacggccgtttattactgtgcagcagagtatctagggaatctacggcactttaggggggaccactggggcaaagggacccaggtcaccgtctcctca

SEQ ID NO: 83 - protein, 8 aa, Artificial sequence
GLTLGYYA

SEQ ID NO: 84 - DNA, 24 bp, Artificial sequence
  source 1..24: mol_type = other DNA
ggattgactctgggttattatgcc

SEQ ID NO: 85 - protein, 8 aa, Artificial sequence
ISASGGMT

SEQ ID NO: 86 - DNA, 24 bp, Artificial sequence
  source 1..24: mol_type = other DNA
attagcgcgagtggtggtatgaca

SEQ ID NO: 87 - protein, 15 aa, Artificial sequence
AAEYLGNLRHFRGDH

SEQ ID NO: 88 - DNA, 45 bp, Artificial sequence
  source 1..45: mol_type = other DNA
gcagcagagtatctagggaatctacggcactttaggggggaccac

SEQ ID NO: 89 - protein, 125 aa, Artificial sequence
QVQLQESGGGLVQPGGSLRLSCAASGRVFSSDAMGWFRQAPGNEREFVAAIIWSGSSTHYADSVKGRFTISRDNAKNTGYLQMNSLKPEDTAVYYCAVDTRPPYGLRNANRYDYWGQGTQVTVSS

SEQ ID NO: 90 - DNA, 375 bp, Artificial sequence
  source 1..375: mol_type = other DNA
caggtgcagctgcaggagtctgggggaggcttggtgcagcctggggggtctctgagactctcctgtgcagcctctggacgcgtcttcagtagcgatgccatgggctggttccgccaggctccagggaacgagcgtgagtttgtagcagctattatctggagtggtagtagcacacactatgcagactccgtgaagggccgattcaccatctccagagacaacgccaagaacacggggtatctgcaaatgaacagcctgaaacctgaggacacggccgtttattactgtgcagtagacactcgccctccatacggattgaggaacgcaaaccggtatgactactggggccaggggacccaggtcaccgtctcctca

SEQ ID NO: 91 - protein, 8 aa, Artificial sequence
GRVFSSDA

SEQ ID NO: 92 - DNA, 24 bp, Artificial sequence
  source 1..24: mol_type = other DNA
ggacgcgtcttcagtagcgatgcc

SEQ ID NO: 93 - protein, 8 aa, Artificial sequence
IIWSGSST

SEQ ID NO: 94 - DNA, 24 bp, Artificial sequence
  source 1..24: mol_type = other DNA
attatctggagtggtagtagcaca

SEQ ID NO: 95 - protein, 18 aa, Artificial sequence
AVDTRPPYGLRNANRYDY

SEQ ID NO: 96 - DNA, 54 bp, Artificial sequence; identical to SEQ ID NO: 16
  source 1..54: mol_type = other DNA

SEQ ID NO: 97 - protein, 116 aa, Artificial sequence
QVQLQESGGGLVQPGGSLRLSCAASGFTFSMAVMGWYRQAPGKQRELVATITPGGNTYYVDSVKGRFTISRDNAKKTVVLQMNNLEPEDAAVYYCNRAYDTHYDYWGQGTQVTVSS

SEQ ID NO: 98 - DNA, 348 bp, Artificial sequence
  source 1..348: mol_type = other DNA
caggtgcagctgcaggagtctgggggaggcttggtgcagcctggggggtctctgagactctcctgtgcagcctctggatttacattcagtatggctgttatgggctggtaccgccaggctcctgggaagcagcgcgagttggtcgcaactattactcctggtggtaacacgtactatgtagactccgtgaagggccgattcaccatctccagagacaacgccaagaagacggtggttctgcaaatgaataacctggaacctgaggacgcggccgtctattactgtaatcgagcatatgatacccactacgactactggggccaggggacccaggtcaccgtctcctca

SEQ ID NO: 99 - protein, 8 aa, Artificial sequence
GFTFSMAV

SEQ ID NO: 100 - DNA, 24 bp, Artificial sequence
  source 1..24: mol_type = other DNA
ggatttacattcagtatggctgtt

SEQ ID NO: 101 - protein, 7 aa, Artificial sequence
ITPGGNT

SEQ ID NO: 102 - DNA, 21 bp, Artificial sequence
  source 1..21: mol_type = other DNA
attactcctggtggtaacacg

SEQ ID NO: 103 - protein, 10 aa, Artificial sequence
NRAYDTHYDY

SEQ ID NO: 104 - DNA, 30 bp, Artificial sequence
  source 1..30: mol_type = other DNA
aatcgagcatatgatacccactacgactac

SEQ ID NO: 105 - protein, 121 aa, Artificial sequence
QVQLQESGGGLVQAGGSLTLSCAHSGFDFDDYAVGWFRQAPRKGREGISYIRGSDGLTYYADSVKGRFTISRDNAKNLLYLQMNTLEPTDTAVYYCDPKGSTGWNPSGDSWGQGTQVTVSS

SEQ ID NO: 106 - DNA, 363 bp, Artificial sequence
  source 1..363: mol_type = other DNA
caggtgcagctgcaggagtctggaggaggcttggtgcaggctgggggatctctgacgctctcctgtgcacattctggattcgatttcgatgattatgccgtaggctggttccgccaggccccgcggaagggacgtgaggggatctcatatatacgtggtagtgatggtctgacatactatgcagactccgtgaagggccgattcaccatatcgagagacaacgccaagaatctactgtatctgcaaatgaacaccctcgaacccacggacacggccgtgtattactgtgacccgaaggggtctacgggatggaacccttcgggggattcctggggccaggggacccaggtcaccgtctcctca

SEQ ID NO: 107 - protein, 8 aa, Artificial sequence
GFDFDDYA

SEQ ID NO: 108 - DNA, 24 bp, Artificial sequence
  source 1..24: mol_type = other DNA
ggattcgatttcgatgattatgcc

SEQ ID NO: 109 - protein, 8 aa, Artificial sequence
IRGSDGLT

SEQ ID NO: 110 - DNA, 24 bp, Artificial sequence
  source 1..24: mol_type = other DNA
atacgtggtagtgatggtctgaca

SEQ ID NO: 111 - protein, 14 aa, Artificial sequence
DPKGSTGWNPSGDS

SEQ ID NO: 112 - DNA, 42 bp, Artificial sequence
  source 1..42: mol_type = other DNA
gacccgaaggggtctacgggatggaacccttcgggggattcc

SEQ ID NO: 113 - protein, 117 aa, Artificial sequence
QVQLQESGGGLVQPGGSLRLSCAASGSKFSIATMGWYRQAPGKQRDLVASITPGGNTTYADFVKGRFTISRDNAKNTVYLQMNSLKPEDTAVYYCNDFRLAGLRDYWGQGTQVTVSS

SEQ ID NO: 114 - DNA, 351 bp, Artificial sequence
  source 1..351: mol_type = other DNA
caggtgcagctgcaggagtctgggggaggcttggtgcagcctggggggtctctgagactctcctgtgcagcctctggaagcaagttcagtatcgctaccatgggctggtaccgccaggctccagggaagcagcgcgatttggtcgcatctattacgcctggtggtaacacaacctatgcagatttcgtgaagggccgattcaccatctccagagacaacgccaagaacacggtgtatctgcaaatgaacagcctgaaacctgaggacacggccgtctattactgtaatgacttccgtctagctggtctgagggactactggggccaggggacccaggtcaccgtctcctca

SEQ ID NO: 115 - protein, 8 aa, Artificial sequence
GSKFSIAT

SEQ ID NO: 116 - DNA, 24 bp, Artificial sequence
  source 1..24: mol_type = other DNA
ggaagcaagttcagtatcgctacc

SEQ ID NO: 117 - protein, 7 aa, Artificial sequence
ITPGGNT

SEQ ID NO: 118 - DNA, 21 bp, Artificial sequence
  source 1..21: mol_type = other DNA
attacgcctggtggtaacaca

SEQ ID NO: 119 - protein, 11 aa, Artificial sequence
NDFRLAGLRDY

SEQ ID NO: 120 - DNA, 33 bp, Artificial sequence; identical to SEQ ID NO: 56
  source 1..33: mol_type = other DNA

SEQ ID NO: 121 - protein, 122 aa, Artificial sequence
QVQLQESGGGLVQPGGSLRLSCTASGRAFSMYVMGWFRQAPGKEREFVSTISASGGMTYYADSVKGRFTISRDNAKNTVYLEMNSLKPEDTAVYYCAAEYLGNLRHFRGDHWGKGTQVTVSS

SEQ ID NO: 122 - DNA, 366 bp, Artificial sequence
  source 1..366: mol_type = other DNA
caggtgcagctgcaggagtctggaggaggcttggttcagcctggggggtctctgagactctcctgtacagcctctggacgcgccttcagtatgtatgtcatgggctggttccgccaggctccagggaaggagcgtgagtttgtgtcgactattagcgcgagtggtggtatgacatactatgcagactccgtgaagggccgattcaccatctccagagacaacgccaagaacacggtgtatctggaaatgaacagcctgaaacctgaggacacggccgtttattactgtgcagcagagtatctagggaatctacggcactttaggggggaccactggggcaaagggacccaggtcaccgtctcctca

SEQ ID NO: 123 - protein, 8 aa, Artificial sequence
GRAFSMYV

SEQ ID NO: 124 - DNA, 24 bp, Artificial sequence
  source 1..24: mol_type = other DNA
ggacgcgccttcagtatgtatgtc

SEQ ID NO: 125 - protein, 8 aa, Artificial sequence
ISASGGMT

SEQ ID NO: 126 - DNA, 24 bp, Artificial sequence
  source 1..24: mol_type = other DNA
attagcgcgagtggtggtatgaca

SEQ ID NO: 127 - protein, 15 aa, Artificial sequence
AAEYLGNLRHFRGDH

SEQ ID NO: 128 - DNA, 45 bp, Artificial sequence; identical to SEQ ID NO: 88
  source 1..45: mol_type = other DNA

SEQ ID NO: 129 - protein, 124 aa, Artificial sequence
QVQLQESGGGLVQPGGSLRLSCAASGTTLDDYAVGWFRQAPGKEREGVACISASELSTYYADSVKGRFTISRDNAKNTMYLQMNSLKPEDTAVYYCAARVGRIVDVTSTQYQYWGQGTQVTVSS

SEQ ID NO: 130 - DNA, 372 bp, Artificial sequence
  source 1..372: mol_type = other DNA
caggtgcagctgcaggagtctgggggaggcttggtgcagcctggggggtctctgcgactctcctgtgcagcctctgggaccactttggatgattacgccgtaggctggttccgccaggccccaggcaaggagcgcgagggggtcgcatgtattagcgctagtgagcttagcacatattatgcagactccgtgaagggccgattcaccatctccagagacaacgccaaaaacacgatgtatctgcaaatgaacagcctgaaacctgaggacacggccgtttattactgtgcagcccgagttgggagaatagtggacgttactagtacacagtatcagtactggggccaggggacccaggtcaccgtctcctca

SEQ ID NO: 131 - protein, 8 aa, Artificial sequence
GTTLDDYA

SEQ ID NO: 132 - DNA, 24 bp, Artificial sequence
  source 1..24: mol_type = other DNA
gggaccactttggatgattacgcc

SEQ ID NO: 133 - protein, 8 aa, Artificial sequence
ISASELST

SEQ ID NO: 134 - DNA, 24 bp, Artificial sequence
  source 1..24: mol_type = other DNA
attagcgctagtgagcttagcaca

SEQ ID NO: 135 - protein, 17 aa, Artificial sequence
AARVGRIVDVTSTQYQY

SEQ ID NO: 136 - DNA, 51 bp, Artificial sequence
  source 1..51: mol_type = other DNA
gcagcccgagttgggagaatagtggacgttactagtacacagtatcagtac

SEQ ID NO: 137 - protein, 124 aa, Artificial sequence
QVQLQESGGGLVQPGGSLRLSCAASGRTFSSYNMGWFRQAPGQGLEAVAAISRGGGSTYYADSVKGRFTISRDNSKNTLYLQMNSLRAEDTAVYYCADSGARAYSGSYLDFGSWGQGTQVTVSS

SEQ ID NO: 138 - DNA, 372 bp, Artificial sequence
  source 1..372: mol_type = other DNA
caggtgcagctgcaggagtctggaggaggattggtgcagcctgggggctctctgagactctcctgtgcagcctctggacgcaccttcagtagctataacatgggctggttccgccaggctccagggcaggggctcgaggctgtagcagctattagccggggtggtggtagtacatactatgcagactccgtgaagggccgattcaccatctccagagacaacagcaagaacacgttgtatctgcaaatgaacagcctgcgagctgaggacacggccgtttattactgtgcagactcaggagctcgagcctatagtggtagttacctcgactttggttcctggggccaggggacccaggtcaccgtctcctca

SEQ ID NO: 139 - protein, 8 aa, Artificial sequence
GRTFSSYN

SEQ ID NO: 140 - DNA, 24 bp, Artificial sequence
  source 1..24: mol_type = other DNA
ggacgcaccttcagtagctataac

SEQ ID NO: 141 - protein, 8 aa, Artificial sequence
ISRGGGST

SEQ ID NO: 142 - DNA, 24 bp, Artificial sequence
  source 1..24: mol_type = other DNA
attagccggggtggtggtagtaca

SEQ ID NO: 143 - protein, 17 aa, Artificial sequence
ADSGARAYSGSYLDFGS

SEQ ID NO: 144 - DNA, 51 bp, Artificial sequence; identical to SEQ ID NO: 32
  source 1..51: mol_type = other DNA

SEQ ID NO: 145 - protein, 22 aa, Artificial sequence
MLLLVTSLLLCELPHPAFLLIP

SEQ ID NO: 146 - DNA, 66 bp, Artificial sequence
  source 1..66: mol_type = other DNA
atgctgctgctggtgaccagcctgctgctgtgcgagctgccccaccccgcctttctgctgatcccc

SEQ ID NO: 147 - protein, 46 aa, Artificial sequence
TTPAPRPPTPAPTIASQPLSLRPEACRPAAGGAVHTRGLDFACDIY

SEQ ID NO: 148 - DNA, 138 bp, Artificial sequence
  source 1..138: mol_type = other DNA
actaccccagcaccgcggccgcccaccccggctcctaccatcgcctcccagcctctgtccctgcgtccggaggcatgtagacccgcagctggtggggccgtgcatacccggggtcttgacttcgcctgcgatatctac

SEQ ID NO: 149 - protein, 24 aa, Artificial sequence
IWAPLAGTCGVLLLSLVITLYCKR

SEQ ID NO: 150 - DNA, 72 bp, Artificial sequence
  source 1..72: mol_type = other DNA
atttgggcccctctggctggtacttgcggggtcctgctgctttcactcgtgatcactctttactgtaagcgc

SEQ ID NO: 151 - protein, 42 aa, Artificial sequence
GRKKLLYIFKQPFMRPVQTTQEEDGCSCRFPEEEEGGCELRV

SEQ ID NO: 152 - DNA, 126 bp, Artificial sequence
  source 1..126: mol_type = other DNA
ggtcggaagaagctgctgtacatctttaagcaacccttcatgaggcctgtgcagactactcaagaggaggacggctgttcatgccggttcccagaggaggaggaaggcggctgcgaactgcgcgtg

SEQ ID NO: 153 - protein, 110 aa, Artificial sequence
KFSRSADAPAYKQGQNQLYNELNLGRREEYDVLDKRRGRDPEMGGKPRRKNPQEGLYNELQKDKMAEAYSEIGMKGERRRGKGHDGLYQGLSTATKDTYDALHMQALPPR

SEQ ID NO: 154 - DNA, 330 bp, Artificial sequence
  source 1..330: mol_type = other DNA
aaattcagccgcagcgcagatgctccagcctacaagcaggggcagaaccagctctacaacgaactcaatcttggtcggagagaggagtacgacgtgctggacaagcggagaggacgggacccagaaatgggcgggaagccgcgcagaaagaatccccaagagggcctgtacaacgagctccaaaaggataagatggcagaagcctatagcgagattggtatgaaaggggaacgcagaagaggcaaaggccacgacggactgtaccagggactcagcaccgccaccaaggacacctatgacgctcttcacatgcaggccctgccgcctcgg

SEQ ID NO: 155 - protein, 23 aa, Artificial sequence
LEGGGEGRGSLLTCGDVEENPGP

SEQ ID NO: 156 - DNA, 69 bp, Artificial sequence
  source 1..69: mol_type = other DNA
ctcgagggcggcggagagggcagaggaagtcttctaacatgcggtgacgtggaggagaatcccggccct

SEQ ID NO: 157 - DNA, 1179 bp, Artificial sequence
  source 1..1179: mol_type = other DNA
ggctccggtgcccgtcagtgggcagagcgcacatcgcccacagtccccgagaagttggggggaggggtcggcaattgaaccggtgcctagagaaggtggcgcggggtaaactgggaaagtgatgtcgtgtactggctccgcctttttcccgagggtgggggagaaccgtatataagtgcagtagtcgccgtgaacgttctttttcgcaacgggtttgccgccagaacacaggtaagtgccgtgtgtggttcccgcgggcctggcctctttacgggttatggcccttgcgtgccttgaattacttccacctggctgcagtacgtgattcttgatcccgagcttcgggttggaagtgggtgggagagttcgaggccttgcgcttaaggagccccttcgcctcgtgcttgagttgaggcctggcctgggcgctggggccgccgcgtgcgaatctggtggcaccttcgcgcctgtctcgctgctttcgataagtctctagccatttaaaatttttgatgacctgctgcgacgctttttttctggcaagatagtcttgtaaatgcgggccaagatctgcacactggtatttcggtttttggggccgcgggcggcgacggggcccgtgcgtcccagcgcacatgttcggcgaggcggggcctgcgagcgcggccaccgagaatcggacgggggtagtctcaagctggccggcctgctctggtgcctggcctcgcgccgccgtgtatcgccccgccctgggcggcaaggctggcccggtcggcaccagttgcgtgagcggaaagatggccgcttcccggccctgctgcagggagctcaaaatggaggacgcggcgctcgggagagcgggcgggtgagtcacccacacaaaggaaaagggcctttccgtcctcagccgtcgcttcatgtgactccacggagtaccgggcgccgtccaggcacctcgattagttctcgagcttttggagtacgtcgtctttaggttggggggaggggttttatgcgatggagtttccccacactgagtgggtggagactgaagttaggccagcttggcacttgatgtaattctccttggaatttgccctttttgagtttggatcttggttcattctcaagcctcagacagtggttcaaagtttttttcttccatttcaggtgtcgtga

SEQ ID NO: 158 - protein, 23 aa, Artificial sequence
RMLLLVTSLLLCELPHPAFLLIP

SEQ ID NO: 159 - DNA, 69 bp, Artificial sequence
  source 1..69: mol_type = other DNA
aggatgcttctcctggtgacaagccttctgctctgtgagttaccacacccagcattcctcctgatccca

SEQ ID NO: 160 - protein, 335 aa, Artificial sequence
RKVCNGIGIGEFKDSLSINATNIKHFKNCTSISGDLHILPVAFRGDSFTHTPPLDPQELDILKTVKEITGFLLIQAWPENRTDLHAFENLEIIRGRTKQHGQFSLAVVSLNITSLGLRSLKEISDGDVIISGNKNLCYANTINWKKLFGTSGQKTKIISNRGENSCKATGQVCHALCSPEGCWGPEPRDCVSCRNVSRGRECVDKCNLLEGEPREFVENSECIQCHPECLPQAMNITCTGRGPDNCIQCAHYIDGPHCVKTCPAGVMGENNTLVWKYADAGHVCHLCHPNCTYGCTGPGLEGCPTNGPKIPSIATGMVGALLLLLVVALGIGLFM

SEQ ID NO: 161 - DNA, 1005 bp, Artificial sequence
  source 1..1005: mol_type = other DNA
cgcaaagtgtgtaacggaataggtattggtgaatttaaagactcactctccataaatgctacgaatattaaacacttcaaaaactgcacctccatcagtggcgatctccacatcctgccggtggcatttaggggtgactccttcacacatactcctcctctggatccacaggaactggatattctgaaaaccgtaaaggaaatcacagggtttttgctgattcaggcttggcctgaaaacaggacggacctccatgcctttgagaacctagaaatcatacgcggcaggaccaagcaacatggtcagttttctcttgcagtcgtcagcctgaacataacatccttgggattacgctccctcaaggagataagtgatggagatgtgataatttccggaaacaaaaatttgtgctatgcaaatacaataaactggaaaaaactgtttgggacctccggtcagaaaaccaaaattataagcaacagaggtgaaaacagctgcaaggccacaggccaggtctgccatgccttgtgctcccccgagggctgctggggcccggagcccagggactgcgtctcttgccggaatgtcagccgaggcagggaatgcgtggacaagtgcaaccttctggagggtgagccaagggagtttgtggagaactctgagtgcatacagtgccacccagagtgcctgcctcaggccatgaacatcacctgcacaggacggggaccagacaactgtatccagtgtgcccactacattgacggcccccactgcgtcaagacctgcccggcaggagtcatgggagaaaacaacaccctggtctggaagtacgcagacgccggccatgtgtgccacctgtgccatccaaactgcacctacggatgcactgggccaggtcttgaaggctgtccaacgaatgggcctaagatcccgtccatcgccactgggatggtgggggccctcctcttgctgctggtggtggccctggggatcggcctcttcatg